European Patent Application EP 4 506 463 A1, published February 12, 2025. Title: "Method and kit for diagnosis, prognosis, therapy monitoring or outcome prediction assessment of a disease". Applicant: Immagina Biotechnology S.r.l. The sequence listing filed with the application follows.

SEQUENCE LISTING (225 sequences)

SEQ ID NO: 1 - RNA, 16 nt, Homo sapiens
  source 1..16: mol_type = tRNA
agcagagtggcgcagc

SEQ ID NO: 2 - RNA, 16 nt, Homo sapiens
  source 1..16: mol_type = tRNA
agcagagtagcgcagc

SEQ ID NO: 3 - RNA, 31 nt, Homo sapiens
  source 1..31: mol_type = tRNA
gggggtgtagctcagtggtagagcgtgcttc

SEQ ID NO: 4 - RNA, 18 nt, Homo sapiens
  source 1..18: mol_type = tRNA
accaggatggccgagtgg

SEQ ID NO: 5 - RNA, 15 nt, Homo sapiens
  source 1..15: mol_type = tRNA
accaggatggccgag

SEQ ID NO: 6 - RNA, 20 nt, Homo sapiens
  source 1..20: mol_type = tRNA
ggggaattagctcaagtggt

SEQ ID NO: 7 - RNA, 22 nt, Homo sapiens
  source 1..22: mol_type = tRNA
agtggttaggattcggcgctct

SEQ ID NO: 8 - RNA, 18 nt, Homo sapiens
  source 1..18: mol_type = tRNA
ggttaggattcggcgctc

SEQ ID NO: 9 - RNA, 18 nt, Homo sapiens
  source 1..18: mol_type = tRNA
accgggatggccgagtgg

SEQ ID NO: 10 - RNA, 24 nt, Homo sapiens
  source 1..24: mol_type = tRNA
agcagagtggcgcagcggaagcgt

SEQ ID NO: 11 - RNA, 16 nt, Homo sapiens
  source 1..16: mol_type = tRNA
agcagagttgcgcagc

SEQ ID NO: 12 - RNA, 15 nt, Homo sapiens
  source 1..15: mol_type = tRNA
agcagagtggcgcag

SEQ ID NO: 13 - RNA, 23 nt, Homo sapiens
  source 1..23: mol_type = tRNA
ataacccagaggtcgatggatcg

SEQ ID NO: 14 - RNA, 30 nt, Homo sapiens
  source 1..30: mol_type = tRNA
gggggtgtagctcagtggtagagcgtgctt

SEQ ID NO: 15 - RNA, 31 nt, Homo sapiens
  source 1..31: mol_type = tRNA
gggggtgtagctcagtggtagagcgtgcttg

SEQ ID NO: 16 - RNA, 34 nt, Homo sapiens
  source 1..34: mol_type = tRNA
gggggtgtagctcagtggtagagcgcgtgcttgg

SEQ ID NO: 17 - RNA, 34 nt, Homo sapiens
  source 1..34: mol_type = tRNA
gggggtatagctcagcggtagagcgcgtgcttgg

SEQ ID NO: 18 - RNA, 31 nt, Homo sapiens
  source 1..31: mol_type = tRNA
gggggtgtagctcagtggtagagcgcgtgct

SEQ ID NO: 19 - RNA, 13 nt, Homo sapiens
  source 1..13: mol_type = tRNA
ggggatgtagctc

SEQ ID NO: 20 - RNA, 13 nt, Homo sapiens
  source 1..13: mol_type = tRNA
ggggaattagctc

SEQ ID NO: 21 - RNA, 30 nt, Homo sapiens; identical to SEQ ID NO: 14
  source 1..30: mol_type = tRNA

SEQ ID NO: 22 - RNA, 20 nt, Homo sapiens
  source 1..20: mol_type = tRNA
gtttccgtagtgtagtggtt

SEQ ID NO: 23 - RNA, 18 nt, Homo sapiens
  source 1..18: mol_type = tRNA
gtttccgtagtgtagtgg

SEQ ID NO: 24 - RNA, 16 nt, Homo sapiens
  source 1..16: mol_type = tRNA
gtttccgtagtgtagt

SEQ ID NO: 25 - RNA, 17 nt, Homo sapiens
  source 1..17: mol_type = tRNA
gtttccgtagtgtagtg

SEQ ID NO: 26 - RNA, 19 nt, Homo sapiens
  source 1..19: mol_type = tRNA
gtttccgtagtgtagtggt

SEQ ID NO: 27 - RNA, 13 nt, Homo sapiens
  source 1..13: mol_type = tRNA
gtttccgtagtgt

SEQ ID NO: 28 - RNA, 36 nt, Homo sapiens
  source 1..36: mol_type = tRNA
gcgttggtggtatagtggttagcatagctgccttcc

SEQ ID NO: 29 - RNA, 20 nt, Homo sapiens
  source 1..20: mol_type = tRNA
gcgttggtggtatagtggtg

SEQ ID NO: 30 - RNA, 35 nt, Homo sapiens
  source 1..35: mol_type = tRNA
gcgttggtggtatagtggttagcatagctgccttc

SEQ ID NO: 31 - RNA, 34 nt, Homo sapiens
  source 1..34: mol_type = tRNA
gcgttggtggtatagtggttagcatagctgcctt

SEQ ID NO: 32 - RNA, 35 nt, Homo sapiens
  source 1..35: mol_type = tRNA
gcgttggtggtatagtggtaagcatagctgccttc

SEQ ID NO: 33 - RNA, 35 nt, Homo sapiens
  source 1..35: mol_type = tRNA
gcgtttgtggtatagtggtgagcatagctgccttc

SEQ ID NO: 34 - RNA, 36 nt, Homo sapiens
  source 1..36: mol_type = tRNA
gcgtttgtggtatagtggttagcatagctgccttcc

SEQ ID NO: 35 - RNA, 34 nt, Homo sapiens
  source 1..34: mol_type = tRNA
gcgttgtggtatagtggtgagcatagctgccttc

SEQ ID NO: 36 - RNA, 23 nt, Homo sapiens
  source 1..23: mol_type = tRNA
gcgttggtggtatagtggtgagc

SEQ ID NO: 37 - RNA, 34 nt, Homo sapiens
  source 1..34: mol_type = tRNA
gcgttggtggtatagtggtaagcatagctgcctt

SEQ ID NO: 38 - RNA, 20 nt, Homo sapiens
  source 1..20: mol_type = tRNA
gcgtttgtggtatagtggtg

SEQ ID NO: 39 - RNA, 35 nt, Homo sapiens
  source 1..35: mol_type = tRNA
gcgttgtggtatagtggttagcatagctgccttcc

SEQ ID NO: 40 - RNA, 33 nt, Homo sapiens
  source 1..33: mol_type = tRNA
gcgttggtggtatagtggtaagcatagctgcct

SEQ ID NO: 41 - RNA, 33 nt, Homo sapiens
  source 1..33: mol_type = tRNA
gcgttgtggtatagtggtgagcatagctgcctt

SEQ ID NO: 42 - RNA, 23 nt, Homo sapiens
  source 1..23: mol_type = tRNA
gcgttggtggtatagtggttagc

SEQ ID NO: 43 - RNA, 36 nt, Homo sapiens
  source 1..36: mol_type = tRNA
tcccatatggtctagcggttaggattcctggttttc

SEQ ID NO: 44 - RNA, 12 nt, Homo sapiens
  source 1..12: mol_type = tRNA
aggattcggcgc

SEQ ID NO: 45 - RNA, 14 nt, Homo sapiens
  source 1..14: mol_type = tRNA
gcattggtggttca

SEQ ID NO: 46 - RNA, 17 nt, Homo sapiens
  source 1..17: mol_type = tRNA
gcattggtggttcagtg

SEQ ID NO: 47 - RNA, 20 nt, Homo sapiens
  source 1..20: mol_type = tRNA
accgggatggccgagtggtt

SEQ ID NO: 48 - RNA, 20 nt, Homo sapiens
  source 1..20: mol_type = tRNA
accagaatggccgagtggtt

SEQ ID NO: 49 - RNA, 19 nt, Homo sapiens
  source 1..19: mol_type = tRNA
accaggatggccgagtggt

SEQ ID NO: 50 - RNA, 21 nt, Homo sapiens
  source 1..21: mol_type = tRNA
gtttccgtagtgtagtggtta

SEQ ID NO: 51 - RNA, 12 nt, Homo sapiens
  source 1..12: mol_type = tRNA
ggttaggattcg

SEQ ID NO: 52 - RNA, 13 nt, Homo sapiens
  source 1..13: mol_type = tRNA
taggattcggcgc

SEQ ID NO: 53 - RNA, 13 nt, Homo sapiens
  source 1..13: mol_type = tRNA
agtggttaggatt

SEQ ID NO: 54 - RNA, 21 nt, Homo sapiens
  source 1..21: mol_type = tRNA
accagaatggccgagtggtta

SEQ ID NO: 55 - RNA, 17 nt, Homo sapiens
  source 1..17: mol_type = tRNA
accaggatggccgagtg

SEQ ID NO: 56 - RNA, 39 nt, Homo sapiens
  source 1..39: mol_type = tRNA
agcagagtggcgcagcggaagcgtgctgggcccataacc

SEQ ID NO: 57 - RNA, 24 nt, Homo sapiens
  source 1..24: mol_type = tRNA
gtttccgtagtgtagtggttatca

SEQ ID NO: 58 - RNA, 22 nt, Homo sapiens
  source 1..22: mol_type = tRNA
gtttccgtagtgtagtggttat

SEQ ID NO: 59 - RNA, 12 nt, Homo sapiens
  source 1..12: mol_type = tRNA
gtttccgtagtg

SEQ ID NO: 60 - RNA, 14 nt, Homo sapiens
  source 1..14: mol_type = tRNA
gtttccgtagtgta

SEQ ID NO: 61 - RNA, 18 nt, Homo sapiens
  source 1..18: mol_type = tRNA
gcttctgtagtgtagtgg

SEQ ID NO: 62 - RNA, 21 nt, Homo sapiens
  source 1..21: mol_type = tRNA
accgggatggccgagtggtta

SEQ ID NO: 63 - RNA, 24 nt, Homo sapiens
  source 1..24: mol_type = tRNA
agcagagttgcgcagcggaagcgt

SEQ ID NO: 64 - RNA, 22 nt, Homo sapiens
  source 1..22: mol_type = tRNA
agcagagtggcgcagcggaagc

SEQ ID NO: 65 - RNA, 31 nt, Homo sapiens
  source 1..31: mol_type = tRNA
agcagttgcgcagcggaagcgtgctgggccc

SEQ ID NO: 66 - RNA, 20 nt, Homo sapiens
  source 1..20: mol_type = tRNA
agcggaagcgtgctgggccc

SEQ ID NO: 67 - RNA, 22 nt, Homo sapiens
  source 1..22: mol_type = tRNA
ataacccagaggtcgatggatc

SEQ ID NO: 68 - RNA, 15 nt, Homo sapiens
  source 1..15: mol_type = tRNA
ggaagcgtgctgggc

SEQ ID NO: 69 - RNA, 20 nt, Homo sapiens
  source 1..20: mol_type = tRNA
ataacccagaggtcgatgga

SEQ ID NO: 70 - RNA, 16 nt, Homo sapiens
  source 1..16: mol_type = tRNA
ggaagcgtgctgggcc

SEQ ID NO: 71 - RNA, 30 nt, Homo sapiens
  source 1..30: mol_type = tRNA
gggggtgtagctcagtggtagagcgcgtgc

SEQ ID NO: 72 - RNA, 32 nt, Homo sapiens
  source 1..32: mol_type = tRNA
gggggtatagctcagcggtagagcgtgcttgg

SEQ ID NO: 73 - RNA, 33 nt, Homo sapiens
  source 1..33: mol_type = tRNA
gggggtatagctcagcggtagagcgtgcttggc

SEQ ID NO: 74 - RNA, 31 nt, Homo sapiens
  source 1..31: mol_type = tRNA
gggggtatagctcagcggtagagcgcgtgct

SEQ ID NO: 75 - RNA, 30 nt, Homo sapiens
  source 1..30: mol_type = tRNA
gggggtatagctcagcggtagagcgcgtgc

SEQ ID NO: 76 - RNA, 35 nt, Homo sapiens
  source 1..35: mol_type = tRNA
gcgtttgtggtatagtggtaagcatagctgccttc

SEQ ID NO: 77 - RNA, 28 nt, Homo sapiens
  source 1..28: mol_type = tRNA
ggtctagtggttaggattcggcgctctc

SEQ ID NO: 78 - RNA, 19 nt, Homo sapiens
  source 1..19: mol_type = tRNA
ggttaggattcggcgctct

SEQ ID NO: 79 - RNA, 15 nt, Homo sapiens
  source 1..15: mol_type = tRNA
ctagtggttaggatt

SEQ ID NO: 80 - RNA, 19 nt, Homo sapiens
  source 1..19: mol_type = tRNA
accgggatggccgagtggt

SEQ ID NO: 81 - RNA, 18 nt, Homo sapiens
  source 1..18: mol_type = tRNA
accagaatggccgagtgg

SEQ ID NO: 82 - RNA, 20 nt, Homo sapiens
  source 1..20: mol_type = tRNA
gtttccgtagtgtagtggtc

SEQ ID NO: 83 - RNA, 20 nt, Homo sapiens
  source 1..20: mol_type = tRNA
ggccggttagctcagttggt

SEQ ID NO: 84 - RNA, 31 nt, Homo sapiens
  source 1..31: mol_type = tRNA
cacgcgggagaccggggttcgattccccgac

SEQ ID NO: 85 - RNA, 35 nt, Homo sapiens
  source 1..35: mol_type = tRNA
gcgggagaccggggttcgattccccgacggggagc

SEQ ID NO: 86 - RNA, 38 nt, Homo sapiens
  source 1..38: mol_type = tRNA
acgcgggagaccggggttcgattccccgacggggagcc

SEQ ID NO: 87 - RNA, 37 nt, Homo sapiens
  source 1..37: mol_type = tRNA
acgcgggagaccggggttcgtttccccgacggggagc

SEQ ID NO: 88 - RNA, 37 nt, Homo sapiens
  source 1..37: mol_type = tRNA
acgcgggagaccggggttcaattccccgacggggagc

SEQ ID NO: 89 - RNA, 35 nt, Homo sapiens
  source 1..35: mol_type = tRNA
gcgggagaccggggttcgtttccccgacggggagc

SEQ ID NO: 90 - RNA, 39 nt, Homo sapiens
  source 1..39: mol_type = tRNA
cacgcgggagaccggggttcgattccccgacggggagcc

SEQ ID NO: 91 - RNA, 38 nt, Homo sapiens
  source 1..38: mol_type = tRNA
acgcgggagaccggggttcaattccccgacggggagcc

SEQ ID NO: 92 - RNA, 38 nt, Homo sapiens
  source 1..38: mol_type = tRNA
acgcgggagaccggggttcgtttccccgacggggagcc

SEQ ID NO: 93 - RNA, 37 nt, Homo sapiens
  source 1..37: mol_type = tRNA
acgcgggagaccggggttcggttccccgacggggagc

SEQ ID NO: 94 - RNA, 39 nt, Homo sapiens
  source 1..39: mol_type = tRNA
cacgcgggagaccggggttcaattccccgacggggagcc

SEQ ID NO: 95 - RNA, 35 nt, Homo sapiens
  source 1..35: mol_type = tRNA
gcgggagaccggggttcggttccccgacggggagc

SEQ ID NO: 96 - RNA, 39 nt, Homo sapiens
  source 1..39: mol_type = tRNA
cacgcgggagaccggggttcgtttccccgacggggagcc

SEQ ID NO: 97 - RNA, 32 nt, Homo sapiens
  source 1..32: mol_type = tRNA
tccctggtggtctagtggttaggattcggcgc

SEQ ID NO: 98 - RNA, 33 nt, Homo sapiens
  source 1..33: mol_type = tRNA
tccctggtggtctagtggttaggattcggcgct

SEQ ID NO: 99 - RNA, 35 nt, Homo sapiens
  source 1..35: mol_type = tRNA
tccctggtggtctagtggttaggattcggcgctct

SEQ ID NO: 100 - RNA, 34 nt, Homo sapiens
  source 1..34: mol_type = tRNA
tccctggtggtctagtggttaggattcggcgctc

SEQ ID NO: 101 - RNA, 31 nt, Homo sapiens
  source 1..31: mol_type = tRNA
tccctgtggtctagtggttaggattcggcgc

SEQ ID NO: 102 - RNA, 32 nt, Homo sapiens
  source 1..32: mol_type = tRNA
tccctgtggtctagtggttaggattcggcgct

SEQ ID NO: 103 - RNA, 31 nt, Homo sapiens
  source 1..31: mol_type = tRNA
tccctggtggtctagtggttaggattcggcg

SEQ ID NO: 104 - RNA, 34 nt, Homo sapiens
  source 1..34: mol_type = tRNA
tccctgtggtctagtggttaggattcggcgctct

SEQ ID NO: 105 - RNA, 29 nt, Homo sapiens
  source 1..29: mol_type = tRNA
tccctggtggtctagtggttaggattcgg

SEQ ID NO: 106 - RNA, 33 nt, Homo sapiens
  source 1..33: mol_type = tRNA
tccctgtggtctagtggttaggattcggcgctc

SEQ ID NO: 107 - RNA, 32 nt, Homo sapiens
  source 1..32: mol_type = tRNA
cccctgtggtctagtggttaggattcggcgct

SEQ ID NO: 108 - RNA, 30 nt, Homo sapiens
  source 1..30: mol_type = tRNA
tccctgtggtctagtggttaggattcggcg

SEQ ID NO: 109 - RNA, 28 nt, Homo sapiens
  source 1..28: mol_type = tRNA
tccctgtggtctagtggttaggattcgg

SEQ ID NO: 110 - RNA, 34 nt, Homo sapiens
  source 1..34: mol_type = tRNA
ccctggtggtctagtggttaggattcggcgctct

SEQ ID NO: 111 - RNA, 34 nt, Homo sapiens
  source 1..34: mol_type = tRNA
cccctgtggtctagtggttaggattcggcgctct

SEQ ID NO: 112 - RNA, 33 nt, Homo sapiens
  source 1..33: mol_type = tRNA
cccctgtggtctagtggttaggattcggcgctc

SEQ ID NO: 113 - RNA, 19 nt, Homo sapiens
  source 1..19: mol_type = tRNA
tccctggtggtctagtggt

SEQ ID NO: 114 - RNA, 18 nt, Homo sapiens
  source 1..18: mol_type = tRNA
ccctggtggtctagtggt

SEQ ID NO: 115 - RNA, 35 nt, Homo sapiens
  source 1..35: mol_type = tRNA
tccctggtggtctagtggctaggattcggcgcttt

SEQ ID NO: 116 - RNA, 35 nt, Homo sapiens
  source 1..35: mol_type = tRNA
tcccacatggtctagcggttaggattcctggtttt

SEQ ID NO: 117 - RNA, 34 nt, Homo sapiens
  source 1..34: mol_type = tRNA
tccctgtggtctagtggctaggattcggcgcttt

SEQ ID NO: 118 - RNA, 18 nt, Homo sapiens
  source 1..18: mol_type = tRNA
tcggtagagcatgagact

SEQ ID NO: 119 - RNA, 17 nt, Homo sapiens
  source 1..17: mol_type = tRNA
tcggtagagcatgagac

SEQ ID NO: 120 - RNA, 19 nt, Homo sapiens
  source 1..19: mol_type = tRNA
tcggtagagcatgagactc

SEQ ID NO: 121 - RNA, 24 nt, Homo sapiens
  source 1..24: mol_type = tRNA
agggtcgtgggttcgtgccccacg

SEQ ID NO: 122 - RNA, 32 nt, Homo sapiens
  source 1..32: mol_type = tRNA
agggtcgtgggttcgggccccacgttgggcgc

SEQ ID NO: 123 - RNA, 34 nt, Homo sapiens; identical to SEQ ID NO: 31
  source 1..34: mol_type = tRNA

SEQ ID NO: 124 - RNA, 34 nt, Homo sapiens
  source 1..34: mol_type = tRNA
gcgttggtggtatagtggtgagcatagctgcctt

SEQ ID NO: 125 - RNA, 35 nt, Homo sapiens; identical to SEQ ID NO: 30
  source 1..35: mol_type = tRNA

SEQ ID NO: 126 - RNA, 36 nt, Homo sapiens; identical to SEQ ID NO: 28
  source 1..36: mol_type = tRNA

SEQ ID NO: 127 - RNA, 33 nt, Homo sapiens
  source 1..33: mol_type = tRNA
gcgttggtggtatagtggttagcatagctgcct

SEQ ID NO: 128 - RNA, 30 nt, Homo sapiens
  source 1..30: mol_type = tRNA
gcgttggtggtatagtggttagcatagctg

SEQ ID NO: 129 - RNA, 34 nt, Homo sapiens
  source 1..34: mol_type = tRNA
gcgtttgtggtatagtggtgagcatagctgcctt

SEQ ID NO: 130 - RNA, 34 nt, Homo sapiens
  source 1..34: mol_type = tRNA
gcgtttgtggtatagtggttagcatagctgcctt

SEQ ID NO: 131 - RNA, 33 nt, Homo sapiens
  source 1..33: mol_type = tRNA
gcgttgtggtatagtggttagcatagctgcctt

SEQ ID NO: 132 - RNA, 33 nt, Homo sapiens; identical to SEQ ID NO: 41
  source 1..33: mol_type = tRNA

SEQ ID NO: 133 - RNA, 36 nt, Homo sapiens; identical to SEQ ID NO: 34
  source 1..36: mol_type = tRNA

SEQ ID NO: 134 - RNA, 35 nt, Homo sapiens; identical to SEQ ID NO: 39
  source 1..35: mol_type = tRNA

SEQ ID NO: 135 - RNA, 34 nt, Homo sapiens
  source 1..34: mol_type = tRNA
gcgttgtggtatagtggttagcatagctgccttc

SEQ ID NO: 136 - RNA, 33 nt, Homo sapiens
  source 1..33: mol_type = tRNA
gcgtttgtggtatagtggttagcatagctgcct

SEQ ID NO: 137 - RNA, 32 nt, Homo sapiens
  source 1..32: mol_type = tRNA
gcgttgtggtatagtggttagcatagctgcct

SEQ ID NO: 138 - RNA, 19 nt, Homo sapiens
  source 1..19: mol_type = tRNA
acgcgggaggcccgggttc

SEQ ID NO: 139 - RNA, 15 nt, Homo sapiens
  source 1..15: mol_type = tRNA
agcgcattggatttc

SEQ ID NO: 140 - RNA, 15 nt, Homo sapiens
  source 1..15: mol_type = tRNA
agcgcattggagttc

SEQ ID NO: 141 - RNA, 19 nt, Homo sapiens
  source 1..19: mol_type = tRNA
aatccagcgatccgagttc

SEQ ID NO: 142 - RNA, 15 nt, Homo sapiens
  source 1..15: mol_type = tRNA
ctcggtggaacctcc

SEQ ID NO: 143 - RNA, 28 nt, Homo sapiens
  source 1..28: mol_type = tRNA
ggtagcgtggccgagcggtctaaggctc

SEQ ID NO: 144 - RNA, 29 nt, Homo sapiens
  source 1..29: mol_type = tRNA
ggtagcgtggccgagcggtctaaggctct

SEQ ID NO: 145 - RNA, 27 nt, Homo sapiens
  source 1..27: mol_type = tRNA
ggtagcgtggccgagcggtctaaggcc

SEQ ID NO: 146 - RNA, 33 nt, Homo sapiens
  source 1..33: mol_type = tRNA
ggtagcgtggccgagcggtctaaggctctggat

SEQ ID NO: 147 - RNA, 34 nt, Homo sapiens
  source 1..34: mol_type = tRNA
ggtagcgtggccgagcggtctaaggctctggatt

SEQ ID NO: 148 - RNA, 28 nt, Homo sapiens
  source 1..28: mol_type = tRNA
ggtagcgtggccgagcggtctaaggcct

SEQ ID NO: 149 - RNA, 15 nt, Homo sapiens
  source 1..15: mol_type = tRNA
aggggtcgcgagttc

SEQ ID NO: 150 - RNA, 16 nt, Homo sapiens
  source 1..16: mol_type = tRNA
gccaaggtcgcgggtt

SEQ ID NO: 151 - RNA, 22 nt, Homo sapiens
  source 1..22: mol_type = tRNA
gggtgcgagaggtcccgggttc

SEQ ID NO: 152 - RNA, 21 nt, Homo sapiens
  source 1..21: mol_type = tRNA
gggtgcgagaggtcccgggtt

SEQ ID NO: 153 - RNA, 20 nt, Homo sapiens
  source 1..20: mol_type = tRNA
gctgtgatggccgagtggtt

SEQ ID NO: 154 - RNA, 15 nt, Homo sapiens
  source 1..15: mol_type = tRNA
aagaggtccccggtt

SEQ ID NO: 155 - RNA, 16 nt, Homo sapiens
  source 1..16: mol_type = tRNA
aagaggtccccggttc

SEQ ID NO: 156 - RNA, 21 nt, Homo sapiens
  source 1..21: mol_type = tRNA
ataatctgaaggtcgtgagtt

SEQ ID NO: 157 - RNA, 15 nt, Homo sapiens
  source 1..15: mol_type = tRNA
cataatctgaaggtc

SEQ ID NO: 158 - RNA, 16 nt, Homo sapiens
  source 1..16: mol_type = tRNA
agaaggttgcgtgttc

SEQ ID NO: 159 - RNA, 20 nt, Homo sapiens
  source 1..20: mol_type = tRNA
gatcagaaggttgcgtgttc

SEQ ID NO: 160 - RNA, 15 nt, Homo sapiens
  source 1..15: mol_type = tRNA
atcagaaggttgcgt

SEQ ID NO: 161 - RNA, 15 nt, Homo sapiens
  source 1..15: mol_type = tRNA
agaaggttgcgtgtt

SEQ ID NO: 162 - RNA, 19 nt, Homo sapiens
  source 1..19: mol_type = tRNA
tcggtagagcatgggactc

SEQ ID NO: 163 - RNA, 24 nt, Homo sapiens
  source 1..24: mol_type = tRNA
agggtcgtgggttcgggccccacg

SEQ ID NO: 164 - RNA, 15 nt, Homo sapiens
  source 1..15: mol_type = tRNA
tcggtagagcatgag

SEQ ID NO: 165 - RNA, 16 nt, Homo sapiens
  source 1..16: mol_type = tRNA
aggagatcctgggttc

SEQ ID NO: 166 - RNA, 16 nt, Homo sapiens
  source 1..16: mol_type = tRNA
caggggtcgcgagttc

SEQ ID NO: 167 - RNA, 20 nt, Homo sapiens
  source 1..20: mol_type = tRNA
aaccgaaaggttggtggttc

SEQ ID NO: 168 - RNA, 15 nt, Homo sapiens
  source 1..15: mol_type = tRNA
agtcggtagagcatc

SEQ ID NO: 169 - RNA, 16 nt, Homo sapiens
  source 1..16: mol_type = tRNA
aagaggtccctggttc

SEQ ID NO: 170 - RNA, 17 nt, Homo sapiens
  source 1..17: mol_type = tRNA
caagaggtccccggttc

SEQ ID NO: 171 - RNA, 23 nt, Homo sapiens
  source 1..23: mol_type = tRNA
cataatctgaaggtcgtgagttc

SEQ ID NO: 172 - RNA, 17 nt, Homo sapiens
  source 1..17: mol_type = tRNA
ctgaaggtcgtgagttc

SEQ ID NO: 173 - RNA, 56 nt, synthetic construct
  source 1..56: mol_type = other RNA
  modified_base 56: mod_base = OTHER; note = 3 Fluoro_Uridine
  modified_base 29..31: mod_base = OTHER; note = abasic site
nnnntctccttgcataatcaccaaccatnnnacacgacgctcttccgatctnnnnn

SEQ ID NO: 174 - RNA, 64 nt, synthetic construct
  source 1..64: mol_type = other RNA
  modified_base 29..31: mod_base = OTHER; note = abasic site
  modified_base 64: mod_base = OTHER; note = 3 fluoro uridine
nnnntctccttgcataatcaccaaccatnnnacacgacgctcttccgatctnnnngtaccttgn

SEQ ID NO: 175 - RNA, 64 nt, synthetic construct
  source 1..64: mol_type = other RNA
  modified_base 29..31: mod_base = OTHER; note = abasic site
  modified_base 64: mod_base = OTHER; note = 3 fluoro uridine
nnnntctccttgcataatcaccaaccatnnnacacgacgctcttccgatctnnnntaatgccgn

SEQ ID NO: 176 - RNA, 64 nt, synthetic construct
  source 1..64: mol_type = other RNA
  modified_base 37..39: mod_base = OTHER; note = abasic site
  modified_base 64: mod_base = OTHER; note = 3 fluoro uridine
nnnntgactgactctccttgcataatcaccaaccatnnnacacgacgctcttccgatctnnnnn

SEQ ID NO: 177 - RNA, 64 nt, synthetic construct
  source 1..64: mol_type = other RNA
  modified_base 37..39: mod_base = OTHER; note = abasic site
  modified_base 64: mod_base = OTHER; note = 3 fluoro uridine
nnnngtaccttgtctccttgcataatcaccaaccatnnnacacgacgctcttccgatctnnnnn

SEQ ID NO: 178 - DNA, 59 bp, synthetic construct
  source 1..59: mol_type = other DNA
gtgactggagttcagacgtgtgctcttccgatctnnnnggttggtgattatgcaaggag

SEQ ID NO: 179 - DNA, 33 bp, synthetic construct
  source 1..33: mol_type = other DNA
acactctttccctacacgacgctcttccgatct

SEQ ID NO: 180 - DNA, 21 bp, synthetic construct
  source 1..21: mol_type = other DNA
gtgactggagttcagacgtgt

SEQ ID NO: 181 - DNA, 29 bp, synthetic construct
  source 1..29: mol_type = other DNA
aatgatacggcgaccaccgagatctacac

SEQ ID NO: 182 - DNA, 33 bp, synthetic construct; identical to SEQ ID NO: 179
  source 1..33: mol_type = other DNA

SEQ ID NO: 183 - DNA, 24 bp, synthetic construct
  source 1..24: mol_type = other DNA
caagcagaagacggcatacgagat

SEQ ID NO: 184 - DNA, 34 bp, synthetic construct
  source 1..34: mol_type = other DNA
gtgactggagttcagacgtgtgctcttccgatct

SEQ ID NO: 185 - RNA, 48 nt, synthetic construct
  source 1..48: mol_type = other RNA
  modified_base 25..27: mod_base = OTHER; note = abasic site
tctccttgcataatcaccaaccatnnngatggaagacgccaaaaacat

SEQ ID NO: 186 - DNA, 35 bp, synthetic construct
  source 1..35: mol_type = other DNA
gtgactggagttcagacgatggttggtgattatgc

SEQ ID NO: 187 - DNA, 22 bp, synthetic construct
  source 1..22: mol_type = other DNA
agacgccaaaaacataaatgga

SEQ ID NO: 188 - DNA, 21 bp, synthetic construct
  source 1..21: mol_type = other DNA
tatgcaaggagactcctactc

SEQ ID NO: 189 - DNA, 21 bp, synthetic construct
  source 1..21: mol_type = other DNA
tatgcaaggagactcctactt

SEQ ID NO: 190 - DNA, 20 bp, synthetic construct
  source 1..20: mol_type = other DNA
aaaacatacgcgaaaggtcc

SEQ ID NO: 191 - DNA, 19 bp, synthetic construct
  source 1..19: mol_type = other DNA
tgcaaggagaggtgtttcc

SEQ ID NO: 192 - DNA, 21 bp, synthetic construct
  source 1..21: mol_type = other DNA
aaaacatacgcagaaggtcct

SEQ ID NO: 193 - DNA, 19 bp, synthetic construct
  source 1..19: mol_type = other DNA
aaggagaggtggttccact

SEQ ID NO: 194 - DNA, 19 bp, synthetic construct
  source 1..19: mol_type = other DNA
aaaacattccctggtggtc

SEQ ID NO: 195 - DNA, 18 bp, synthetic construct
  source 1..18: mol_type = other DNA
caaggagaagcgccgaat

SEQ ID NO: 196 - DNA, 19 bp, synthetic construct
  source 1..19: mol_type = other DNA
aaaacatacgcgggagacc

SEQ ID NO: 197 - DNA, 17 bp, synthetic construct
  source 1..17: mol_type = other DNA
aaggagagctccccgtc

SEQ ID NO: 198 - DNA, 20 bp, synthetic construct
  source 1..20: mol_type = other DNA
ccaaaaacatgtttccgtag

SEQ ID NO: 199 - DNA, 20 bp, synthetic construct
  source 1..20: mol_type = other DNA
tatgcaaggagatgataacc

SEQ ID NO: 200 - DNA, 18 bp, synthetic construct
  source 1..18: mol_type = other DNA
gccaaaacataccgggat

SEQ ID NO: 201 - DNA, 18 bp, synthetic construct
  source 1..18: mol_type = other DNA
tatgcaaggagaccactc

SEQ ID NO: 202 - DNA, 19 bp, synthetic construct
  source 1..19: mol_type = other DNA
ccaaaaacatgcgtttgtg

SEQ ID NO: 203 - DNA, 18 bp, synthetic construct
  source 1..18: mol_type = other DNA
caaggagagaaggcagct

SEQ ID NO: 204 - DNA, 20 bp, synthetic construct
  source 1..20: mol_type = other DNA
gatggaagacgccaaaaaca

SEQ ID NO: 205 - DNA, 19 bp, synthetic construct
  source 1..19: mol_type = other DNA
gtgactggagttcagacga

SEQ ID NO: 206 - DNA, 29 bp, synthetic construct
  source 1..29: mol_type = other DNA
aatgatacggcgaccaccgagatctacac

SEQ ID NO: 207 - DNA, 24 bp, synthetic construct
  source 1..24: mol_type = other DNA
caagcagaagacggcatacgagat

SEQ ID NO: 208 - RNA, 40 nt, Homo sapiens
  source 1..40: mol_type = tRNA
gaaatcaggagctcagccatgtctctgtggcgcaatcggc

SEQ ID NO: 209 - RNA, 40 nt, Homo sapiens
  source 1..40: mol_type = tRNA
ttcgaacccacccagaggcgtcgctgatattttataactc

SEQ ID NO: 210 - RNA, 17 nt, Homo sapiens
  source 1..17: mol_type = mRNA
caacatgaaactaccta

SEQ ID NO: 211 - RNA, 23 nt, Homo sapiens
  source 1..23: mol_type = mRNA
acccaacaacatgaaactaccta

SEQ ID NO: 212 - RNA, 38 nt, Homo sapiens
  source 1..38: mol_type = other RNA
acgaaggtggttttctcagggcgaggcttatccattgc

SEQ ID NO: 213 - RNA, 38 nt, Homo sapiens
  source 1..38: mol_type = other RNA
gcaatggataagcctcgccctgagaaaaccaccttcgt

SEQ ID NO: 214 - RNA, 35 nt, Homo sapiens
  source 1..35: mol_type = other RNA
aaccaggccngaccctgcttagcttccgagatcag

SEQ ID NO: 215 - RNA, 31 nt, Homo sapiens
  source 1..31: mol_type = other RNA
caggcccgaccctgcttagcttccgagatca

SEQ ID NO: 216 - RNA, 29 nt, Homo sapiens
  source 1..29: mol_type = other RNA
ggcccgaccctgcttagcttccgagatca

SEQ ID NO: 217 - RNA, 35 nt, Homo sapiens
  source 1..35: mol_type = tRNA
gcgagaggtcccgggttcaaatcccggacgagccc

SEQ ID NO: 218 - RNA, 31 nt, Homo sapiens; identical to SEQ ID NO: 18
  source 1..31: mol_type = tRNA

SEQ ID NO: 219 - RNA, 39 nt, Homo sapiens
  source 1..39: mol_type = tRNA
acgcgggagaccggggttcgattccccgacggggagcca

SEQ ID NO: 220 - RNA, 36 nt, Homo sapiens
  source 1..36: mol_type = tRNA
tccctggtggtctagtggttaggattcggcgctctc

SEQ ID NO: 221 - RNA, 35 nt, Homo sapiens
  source 1..35: mol_type = tRNA
gcattggtggttcagtggtagaattctcgcctgcc

SEQ ID NO: 222 - DNA, 21 bp, synthetic construct
  source 1..21: mol_type = other DNA
ccaaaacattccctggtggtc

SEQ ID NO: 223 - DNA, 19 bp, synthetic construct
  source 1..19: mol_type = other DNA
aaggagagagagcgccgaa

SEQ ID NO: 224 - DNA, 20 bp, synthetic construct
  source 1..20: mol_type = other DNA
ccaaaacatgggggtgtagc

SEQ ID NO: 225 - DNA, 16 bp, synthetic construct
  source 1..16: mol_type = other DNA
aaggagagcacgcgct